European Patent Application EP 4 215 211 A1, published July 26, 2023. Title: Regulator for tumor immune microenvironment (TIME), and the use thereof for prevention, treatment or diagnosis. Applicant: The University of Tokyo. The sequence listing filed with the application follows.

SEQUENCE LISTING (48 sequences)

SEQ ID NO: 1 - protein, 11 aa, Mus musculus
GYSIASDYAWN

SEQ ID NO: 2 - protein, 16 aa, Mus musculus
YINYSGSTGYNPSLKS

SEQ ID NO: 3 - protein, 5 aa, Mus musculus
FEAGY

SEQ ID NO: 4 - protein, 11 aa, Mus musculus
KASQDINRYLS

SEQ ID NO: 5 - protein, 7 aa, Mus musculus
RANRLVD

SEQ ID NO: 6 - protein, 9 aa, Mus musculus
LQYNEFPLT

SEQ ID NO: 7 - protein, 10 aa, Mus musculus
GYTFTDHAIH

SEQ ID NO: 8 - protein, 17 aa, Mus musculus
YISPGNGDLKYNEKFKG

SEQ ID NO: 9 - protein, 4 aa, Mus musculus
GWTL

SEQ ID NO: 10 - protein, 17 aa, Mus musculus
KSSQSLLYRSNQKNYLV

SEQ ID NO: 11 - protein, 7 aa, Mus musculus
WAFTRES

SEQ ID NO: 12 - protein, 9 aa, Mus musculus
QQHYSYPWT

SEQ ID NO: 13 - protein, 11 aa, Mus musculus
GYSITSDYAWN

SEQ ID NO: 14 - protein, 16 aa, Mus musculus
YINYSGSTGYNPSLKS

SEQ ID NO: 15 - protein, 5 aa, Mus musculus
FEAGY

SEQ ID NO: 16 - protein, 11 aa, Mus musculus
KASQDINSYLS

SEQ ID NO: 17 - protein, 7 aa, Mus musculus
RANRLVD

SEQ ID NO: 18 - protein, 9 aa, Mus musculus
LQYYEFPLT

SEQ ID NO: 19 - protein, 170 aa, Mus musculus
MRVLILLWLFTAFPGILSDVQLQESGPGLVKPSQSLSLTCTATGYSIASDYAWNWIRQFPGNKLEWMGYINYSGSTGYNPSLKSRISITRDTSKNQFFLQLNSVTTEDTATYYCARFEAGYWGQGTTLTVSSAKTTPPSVYPLAPGSAAQTNSMVTLGCLVKGYFPEPVT

SEQ ID NO: 20 - protein, 170 aa, Mus musculus
MEWSWVFLFFLSVTTGVHSEVQLQQSDAELVKPGASVKISCKASGYTFTDHAIHWAKQKPEQGLEWIGYISPGNGDLKYNEKFKGKATLTTDKSSSTAYMQLNSLTSEDSAVYFCKSGWTLWGQGTTLTVSSAKTTPPSVYPLAPGSAAQTNSMVTLGCLVKGYFPEPVT

SEQ ID NO: 21 - protein, 170 aa, Mus musculus
MRVLILLWLFTAFPGILSDVQLQESGPGLVKPSQSLSLTCTATGYSITSDYAWNWIRQFPGNKLEWMGYINYSGSTGYNPSLKSRISITRDTSKNKFFLQLNSVTTEDTATYYCARFEAGYWGQGTTLTVSSAKTTPPSVYPLAPGSAAQTNSMVTLGCLVKGYFPEPVT

SEQ ID NO: 22 - protein, 159 aa, Mus musculus
MDMRTPAQFLGILLLWFPGIKCDIKMTQSPSSMSASLGERVTITCKASQDINRYLSWFQQKPGKSPKTLIYRANRLVDGVPSRFSGSGSGQDYSLTISSLEYGDMGIYYCLQYNEFPLTFGAGTKLELKRADAAPTVSIFPPSSEQLTSGGASVVCFLN

SEQ ID NO: 23 - protein, 163 aa, Mus musculus
MDSQAQVLMLLLLWVSGTCGDIVMSQSPSSPVVSVGEKVTMSCKSSQSLLYRSNQKNYLVWYQLKPGQSPKLLIYWAFTRESGVPDRFTGSGSGTDFTLTISSVKAEDLAVYYCQQHYSYPWTFGGGTKLEVKRADAAPTVSIFPPSSEQLTSGGASVVCFLN

SEQ ID NO: 24 - protein, 159 aa, Mus musculus
MDMRTPAQFLGILLLWFPGIKCDIKMTQSPSSMYASLGERVTFTCKASQDINSYLSWFQQKPGKSPKTLIYRANRLVDGVPSRFSGSGSGQDYSLTISSLDYEDMGIYYCLQYYEFPLTFGAGTKLELKRADAAPTVSIFPPSSEQLTSGGASVVCFLN

SEQ ID NO: 25 - protein, 20 aa, Homo sapiens
EDGVTPYMIFFKDGLEMEKC

SEQ ID NO: 26 - DNA, 20 bp, Artificial Sequence
  Synthetic primer
ctcatgaccacagtccatgc

SEQ ID NO: 27 - DNA, 20 bp, Artificial Sequence
  Synthetic primer
cacattgggggtaggaacac

SEQ ID NO: 28 - DNA, 24 bp, Artificial Sequence
  Synthetic primer
tcataccaggagaaagtcaacctc

SEQ ID NO: 29 - DNA, 24 bp, Artificial Sequence
  Synthetic primer
gtatatgggctcataccagggttt

SEQ ID NO: 30 - DNA, 20 bp, Artificial Sequence
  Synthetic primer
agaccatggctgggattcac

SEQ ID NO: 31 - DNA, 20 bp, Artificial Sequence
  Synthetic primer
agcttcagggtcaaggcaag

SEQ ID NO: 32 - DNA, 20 bp, Artificial Sequence
  Synthetic primer
tccagagcttgagtgtgacg

SEQ ID NO: 33 - DNA, 22 bp, Artificial Sequence
  Synthetic primer
tcagttagccttgcctttgttc

SEQ ID NO: 34 - DNA, 22 bp, Artificial Sequence
  Synthetic primer
gacaccctcatgagaaccaagc

SEQ ID NO: 35 - DNA, 22 bp, Artificial Sequence
  Synthetic primer
gttaaggcagctgtggaggaag

SEQ ID NO: 36 - DNA, 20 bp, Artificial Sequence
  Synthetic primer
gtggaccttccaggatgagg

SEQ ID NO: 37 - DNA, 20 bp, Artificial Sequence
  Synthetic primer
cggagcctgtagtgcagttg

SEQ ID NO: 38 - DNA, 20 bp, Artificial Sequence
  Synthetic DNA
cgggcggaaaaggccgacgc

SEQ ID NO: 39 - DNA, 20 bp, Artificial Sequence
  Synthetic DNA
aggcccgccatttcccgcgc

SEQ ID NO: 40 - protein, 20 aa, Homo sapiens
MYRMQLLSCIALSLALVTNS

SEQ ID NO: 41 - DNA, 30 bp, Artificial Sequence
  Synthetic primer
aagcagtggtatcaacgcagagtacatggg

SEQ ID NO: 42 - DNA, 22 bp, Artificial Sequence
  Synthetic primer
ttgtcgttcactgccatcaatc

SEQ ID NO: 43 - DNA, 21 bp, Artificial Sequence
  Synthetic primer
ggggtaccatctaccttccag

SEQ ID NO: 44 - DNA, 20 bp, Artificial Sequence
  Synthetic primer
agctgggaaggtgtgcacac

SEQ ID NO: 45 - DNA, 22 bp, Artificial Sequence
  Synthetic primer
aagcagtggtatcaacgcagag

SEQ ID NO: 46 - DNA, 24 bp, Artificial Sequence
  Synthetic primer
acattgatgtctttggggtagaag

SEQ ID NO: 47 - DNA, 20 bp, Artificial Sequence
  Synthetic primer
atcgtacacaccagtgtggc

SEQ ID NO: 48 - DNA, 20 bp, Artificial Sequence
  Synthetic primer
gggatccagagttccaggtc